European Patent Specification EP 3 966 568 B1, published July 3, 2024. Title: RESPIRATORY INFECTION DETECTION AND CLASSIFICATION. Applicant: AROCELL AB. The sequence listing filed with the application follows.

SEQUENCE LISTING (28 sequences)

SEQ ID NO: 1 - protein, 10 aa, Homo sapiens
GEAVAARKLF

SEQ ID NO: 2 - protein, 10 aa, Homo sapiens
NCPVPGKPGE

SEQ ID NO: 3 - protein, 10 aa, Homo sapiens
PVPGKPGEAV

SEQ ID NO: 4 - protein, 12 aa, Homo sapiens
NCPVPGKPGEAV

SEQ ID NO: 5 - protein, 5 aa, Artificial Sequence
  VH CDR region of monoclonal anti-TK1 antibody
DYEMH

SEQ ID NO: 6 - protein, 17 aa, Artificial Sequence
  VH CDR region of monoclonal anti-TK1 antibody
AIHPGYGGTAYNQKFKG

SEQ ID NO: 7 - protein, 7 aa, Artificial Sequence
  VH CDR region of monoclonal anti-TK1 antibody
FITKFDY

SEQ ID NO: 8 - protein, 16 aa, Artificial Sequence
  VL CDR region of monoclonal anti-TK1 antibody
KSSQSLLDSDGKTFLN

SEQ ID NO: 9 - protein, 7 aa, Artificial Sequence
  VL CDR region of monoclonal anti-TK1 antibody
LVSKLDS

SEQ ID NO: 10 - protein, 9 aa, Artificial Sequence
  VL CDR region of monoclonal anti-TK1 antibody
WQGTHFPWT

SEQ ID NO: 11 - protein, 6 aa, Artificial Sequence
  VH CDR region of monoclonal anti-TK1 antibody
SGYSWH

SEQ ID NO: 12 - protein, 16 aa, Artificial Sequence
  VH CDR region of monoclonal anti-TK1 antibody
YIHYSGSTTYNPSLKG

SEQ ID NO: 13 - protein, 10 aa, Artificial Sequence
  VH CDR region of monoclonal anti-TK1 antibody
WGTGHWYFDV

SEQ ID NO: 14 - protein, 14 aa, Artificial Sequence
  VL CDR region of monoclonal anti-TK1 antibody
RSSTGAVTTTNYAN

SEQ ID NO: 15 - protein, 7 aa, Artificial Sequence
  VL CDR region of monoclonal anti-TK1 antibody
GTNNRVP

SEQ ID NO: 16 - protein, 9 aa, Artificial Sequence
  VL CDR region of monoclonal anti-TK1 antibody
ALWYSNHWV

SEQ ID NO: 17 - protein, 17 aa, Artificial Sequence
  VH CDR region of monoclonal anti-TK1 antibody
AILPGSGGTAYNQKFKG

SEQ ID NO: 18 - protein, 7 aa, Artificial Sequence
  VH CDR region of monoclonal anti-TK1 antibody
LITTFDY

SEQ ID NO: 19 - protein, 16 aa, Artificial Sequence
  VL CDR region of monoclonal anti-TK1 antibody
KSSQSLLDSDGKTYLN

SEQ ID NO: 20 - protein, 15 aa, Homo sapiens
KPGEAVAARKLFAPQ

SEQ ID NO: 21 - protein, 23 aa, Homo sapiens
AYTKRLGTEKEVEVIGGADKYHS

SEQ ID NO: 22 - protein, 185 aa, Artificial Sequence
  VH domain of anti-TK1 antibody
METGLRWLLLVAVLKGVQCQEQLEESGGDLVKPEGSLTLTCTASRFSFSSSYWICWVRQAPGKGLEWIACIYAGDSGSSYYASWAKGRFTVSKTSSTTVTLQTTSLTAADTATYFCARASVGAAYDYFALWGPGTLVTVSSGQPKAPSVFPLAPCCGDTPSSTVTLGCLVKGYLPEPVTVTWNSG

SEQ ID NO: 23 - protein, 236 aa, Artificial Sequence
  VL domain of anti-TK1 antibody
MDTRAPTQLLGLLLLWLPGARCALVMTQTPASVEAAMGGTVTIKCQASEDVSSHLAWYQQRPGQPPKLLIYGASDLASGVPSRFTGSGSGTQFTLAISDLECADAATYYCQGYYYISDSPYVFGGGTEVVVKGDPVAPTVLIFPPAADQVATGTVTIVCVANKYFPDVTVTWEVDGTTQTTGIENSKTPQNSADCTYNLSSTLTLTSTQYNSHKEYTCKVTQGTTSVVQSFNRGDC

SEQ ID NO: 24 - protein, 187 aa, Artificial Sequence
  VH domain of anti-TK1 antibody
METGLRWLLLVAVLKGVQCQSLEESGGGLVQPEGSLTLTCTASGFSFSSGYDMCWVRQTPGKGLEWIACISVDSDGVTYYASWAKGRFTISKTSSTTVTLQMTSLTAADTATYFCARGYESSSGVYIPYFTLWGPGTLVTVSSGQPKAPSVFPLAPCCGDTPSSTVTLGCLVKGYLPEPVTVTWNSG

SEQ ID NO: 25 - protein, 238 aa, Artificial Sequence
  VL domain of anti-TK1 antibody
MDMRAPTQLLGLLLLWLPGARCADIVLTQTPASVEAAVGGTVTIKCQASQSIYSYLAWYQHKPGQPPKLLIYKASTLASGVPSRFKGSGSGTEYTLTISDLECADAATYYCQHYYYSSTSGGGVFGGGTEVVVKGDPVAPTVLIFPPAADQVATGTVTIVCVANKYFPDVTVTWEVDGTTQTTGIENSKTPQNSADCTYNLSSTLTLTSTQYNSHKEYTCKVTQGTTSVVQSFNRGDC

SEQ ID NO: 26 - protein, 179 aa, Artificial Sequence
  VH domain of anti-TK1 antibody
METGLRWLLLVAVLKGVQCQSLEESGGRLVTPGTPLTLTCTASGFSLSNYYMSWVRQAPGKGLEWIGIIYGDDNTYCANWTKGRFTISKTSTTVDLTITSPTTEDTATYFCARGPDYIAAKMDIWGPGTLVTVSLGQPKAPSVFPLAPCCGDTPSSTVTLGCLVKGYLPEPVTVTWNSG

SEQ ID NO: 27 - protein, 239 aa, Artificial Sequence
  VL domain of anti-TK1 antibody
MDTRAPTQLLGLLLLWLPGARCDVVMTQTPASVEAAVGGTVTIKCQASQSISGYLSWYQQKPGQRPKLLIYRASTLESGVPSRFKGSGSGTEFTLTISDLECADAATYYCQCTYGSSTFSSYGNAFGGGTEVVVKGDPVAPTVLIFPPAADQVATGTVTIVCVANKYFPDVTVTWEVDGTTQTTGIENSKTPQNSADCTYNLSSTLTLTSTQYNSHKEYTCKVTQGTTSVVQSFNRGDC

SEQ ID NO: 28 - protein, 234 aa, Homo sapiens
MSCINLPTVLPGSPSKTRGQIQVILGPMFSGKSTELMRRVRRFQIAQYKCLVIKYAKDTRYSSSFCTHDRNTMEALPACLLRDVAQEALGVAVIGIDEGQFFPDIVEFCEAMANAGKTVIVAALDGTFQRKPFGAILNLVPLAESVVKLTAVCMECFREAAYTKRLGTEKEVEVIGGADKYHSVCRLCYFKKASGQPAGPDNKENCPVPGKPGEAVAARKLFAPQQILQCSPAN